European Patent Specification EP 3 931 348 B1, published August 9, 2023. Title: OLIGONUCLEOTIDE FORMULATION METHOD. Applicant: Roche Innovation Center Copenhagen A/S. The sequence listing filed with the application follows.

SEQUENCE LISTING (20 sequences)

SEQ ID NO: 1 - DNA, 15 bp, artificial
  Oligonucleotide base sequence
cagcgtaaagagagg

SEQ ID NO: 2 - DNA, 16 bp, artificial
  Oligonucleotide base sequence
ctcccaacgtgcgcca

SEQ ID NO: 3 - DNA, 16 bp, artificial
  Oligonucleotide base sequence
cagcgtaaagagaggt

SEQ ID NO: 4 - DNA, 15 bp, artificial
  Oligonucleotide base sequence
cagcgtaaagagagg

SEQ ID NO: 5 - DNA, 15 bp, artificial
  Oligonucleotide base sequence
cagcgtaaagagagg

SEQ ID NO: 6 - DNA, 19 bp, artificial
  Oligonucleotide base sequence
  misc_feature (1)..(19): n is a, c, g, or t
nnnnnnnnnnnnnnnnnnn

SEQ ID NO: 7 - DNA, 12 bp, artificial
  Oligonucleotide base sequence
acgtctcgtagt

SEQ ID NO: 8 - DNA, 20 bp, artificial
  Oligonucleotide base sequence
gcctcagtctgcttcgcacc

SEQ ID NO: 9 - DNA, 15 bp, artificial
  Oligonucleotide base sequence
gctgtgtgagcttgg

SEQ ID NO: 10 - DNA, 14 bp, artificial
  Oligonucleotide base sequence
gcgtaaagagaggt

SEQ ID NO: 11 - DNA, 17 bp, artificial
  Oligonucleotide base sequence
cacgaaccactgaacaa

SEQ ID NO: 12 - DNA, 16 bp, artificial
  Oligonucleotide base sequence
cagcgtaaagagaggt

SEQ ID NO: 13 - DNA, 20 bp, artificial
  Oligonucleotide base sequence
atgtgtctcttctcttcgcc

SEQ ID NO: 14 - DNA, 20 bp, artificial
  Oligonucleotide base sequence
agacaccaataacattagca

SEQ ID NO: 15 - DNA, 20 bp, artificial
  Oligonucleotide base sequence
gctgattagagagaggtccc

SEQ ID NO: 16 - DNA, 16 bp, artificial
  Oligonucleotide base sequence
aatgctacaaaaccca

SEQ ID NO: 17 - DNA, 21 bp, artificial
  Oligonucleotide base sequence
cagaacaaatggcactagtaa

SEQ ID NO: 18 - DNA, 16 bp, artificial
  Oligonucleotide base sequence
ttgaagatgtagatgt

SEQ ID NO: 19 - DNA, 20 bp, artificial
  Oligonucleotide base sequence
agacaccaataacattagca

SEQ ID NO: 20 - DNA, 15 bp, artificial
  Oligonucleotide base sequence
agttataatccagct